European Patent Application EP 4 190 804 A1, published June 7, 2023. Title: Immune Synapse-Stabilizing Chimeric Antigen Receptor(CAR) T Cell. Applicant: TICAROS CO., LTD. The sequence listing filed with the application follows.

SEQUENCE LISTING (44 sequences)

SEQ ID NO: 1 - protein, 185 aa, Artificial Sequence
  CD99
MARGAALALLLFGLLGVLVAAPDGGFDLSDALPDNENKKPTAIPKKPSAGDDFDLGDAVVDGENDDPRPPNPPKPMPNPNPNHPSSSGSFSDADLADGVSGGEGKGGSDGGGSHRKEGEEADAPGVIPGIVGAVVVAVAGAISSFIAYQKKKLCFKENAEQGEVDMESHRNANAEPAVQRTLLEK

SEQ ID NO: 2 - DNA, 558 bp, Artificial Sequence
  CD99
atggcccgcggggctgcgctggcgctgctgctcttcggcctgctgggtgttctggtcgccgccccggatggtggtttcgatttatccgatgcccttcctgacaatgaaaacaagaaacccactgcaatccccaagaaacccagtgctggggatgactttgacttaggagatgctgttgttgatggagaaaatgacgacccacgaccaccgaacccacccaaaccgatgccaaatccaaaccccaaccaccctagttcctccggtagcttttcagatgctgaccttgcggatggcgtttcaggtggagaaggaaaaggaggcagtgatggtggaggcagccacaggaaagaaggggaagaggccgacgccccaggcgtgatccccgggattgtgggggctgtcgtggtcgccgtggctggagccatctctagcttcattgcttaccagaaaaagaagctatgcttcaaagaaaatgcagaacaaggggaggtggacatggagagccaccggaatgccaacgcagagccagctgttcagcgtactcttttagagaaatag

SEQ ID NO: 3 - protein, 25 aa, Artificial Sequence
  CD99 TM
APGVIPGIVGAVVVAVAGAISSFIA

SEQ ID NO: 4 - DNA, 75 bp, Artificial Sequence
  CD99 TM
gccccaggcgtgatccccgggattgtgggggctgtcgtggtcgccgtggctggagccatctctagcttcattgct

SEQ ID NO: 5 - protein, 100 aa, Artificial Sequence
  CD99 EC
DGGFDLSDALPDNENKKPTAIPKKPSAGDDFDLGDAVVDGENDDPRPPNPPKPMPNPNPNHPSSSGSFSDADLADGVSGGEGKGGSDGGGSHRKEGEEAD

SEQ ID NO: 6 - DNA, 300 bp, Artificial Sequence
  CD99 EC
gatggtggtttcgatttatccgatgcccttcctgacaatgaaaacaagaaacccactgcaatccccaagaaacccagtgctggggatgactttgacttaggagatgctgttgttgatggagaaaatgacgacccacgaccaccgaacccacccaaaccgatgccaaatccaaaccccaaccaccctagttcctccggtagcttttcagatgctgaccttgcggatggcgtttcaggtggagaaggaaaaggaggcagtgatggtggaggcagccacaggaaagaaggggaagaggccgac

SEQ ID NO: 7 - protein, 58 aa, Artificial Sequence
  CD99 58EC
DDPRPPNPPKPMPNPNPNHPSSSGSFSDADLADGVSGGEGKGGSDGGGSHRKEGEEAD

SEQ ID NO: 8 - DNA, 174 bp, Artificial Sequence
  CD99 58EC
gacgacccacgaccaccgaacccacccaaaccgatgccaaatccaaaccccaaccaccctagttcctccggtagcttttcagatgctgaccttgcggatggcgtttcaggtggagaaggaaaaggaggcagtgatggtggaggcagccacaggaaagaaggggaagaggccgac

SEQ ID NO: 9 - protein, 45 aa, Artificial Sequence
  CD99 45EC
NPNPNHPSSSGSFSDADLADGVSGGEGKGGSDGGGSHRKEGEEAD

SEQ ID NO: 10 - DNA, 135 bp, Artificial Sequence
  CD99 45EC
aatccaaaccccaaccaccctagttcctccggtagcttttcagatgctgaccttgcggatggcgtttcaggtggagaaggaaaaggaggcagtgatggtggaggcagccacaggaaagaaggggaagaggccgac

SEQ ID NO: 11 - protein, 35 aa, Artificial Sequence
  CD99 35EC
GSFSDADLADGVSGGEGKGGSDGGGSHRKEGEEAD

SEQ ID NO: 12 - DNA, 105 bp, Artificial Sequence
  CD99 35EC
ggtagcttttcagatgctgaccttgcggatggcgtttcaggtggagaaggaaaaggaggcagtgatggtggaggcagccacaggaaagaaggggaagaggccgac

SEQ ID NO: 13 - protein, 11 aa, Artificial Sequence
  CD99 jTM
YQKKKLCFKEN

SEQ ID NO: 14 - DNA, 33 bp, Artificial Sequence
  CD99 jTM
taccagaaaaagaagctatgcttcaaagaaaat

SEQ ID NO: 15 - protein, 41 aa, Artificial Sequence
  CD8 EC
TTTPAPRPPTPAPTIASQPLSLRPEACRPAAGGAVHTRGLD

SEQ ID NO: 16 - DNA, 123 bp, Artificial Sequence
  CD8 EC
accacgacgccagcgccgcgaccaccaacaccggcgcccaccatcgcgtcgcagcccctgtccctgcgcccagaggcgtgccggccagcggcggggggcgcagtgcacacgagggggctggac

SEQ ID NO: 17 - protein, 112 aa, Artificial Sequence
  CD3 zeta intracellular signaling domain(wild type)
RVKFSRSADAPAYQQGQNQLYNELNLGRREEYDVLDKRRGRDPEMGGKPRRKNPQEGLYNELQKDKMAEAYSEIGMKGERRRGKGHDGLYQGLSTATKDTYDALHMQALPPR

SEQ ID NO: 18 - DNA, 336 bp, Artificial Sequence
  CD3 zeta intracellular signaling domain(wild type)
agagtgaagttcagcaggagcgcagacgcccccgcgtaccagcagggccagaaccagctctataacgagctcaatctaggacgaagagaggagtacgatgttttggacaagagacgtggccgggaccctgagatggggggaaagccgagaaggaagaaccctcaggaaggcctgtacaatgaactgcagaaagataagatggcggaggcctacagtgagattgggatgaaaggcgagcgccggaggggcaaggggcacgatggcctttaccagggtctcagtacagccaccaaggacacctacgacgcccttcacatgcaggccctgccccctcgc

SEQ ID NO: 19 - protein, 112 aa, Artificial Sequence
  CD3 zeta intracellular signaling domain(mutant)
RVKFSRSADAPAYKQGQNQLYNELNLGRREEYDVLDKRRGRDPEMGGKPRRKNPQEGLYNELQKDKMAEAYSEIGMKGERRRGKGHDGLYQGLSTATKDTYDALHMQALPPR

SEQ ID NO: 20 - DNA, 336 bp, Artificial Sequence
  CD3 zeta intracellular signaling domain(mutant)
agagtgaagttcagcaggagcgcagacgcccccgcgtacaagcagggccagaaccagctctataacgagctcaatctaggacgaagagaggagtacgatgttttggacaagagacgtggccgggaccctgagatggggggaaagccgagaaggaagaaccctcaggaaggcctgtacaatgaactgcagaaagataagatggcggaggcctacagtgagattgggatgaaaggcgagcgccggaggggcaaggggcacgatggcctttaccagggtctcagtacagccaccaaggacacctacgacgcccttcacatgcaggccctgccccctcgc

SEQ ID NO: 21 - protein, 42 aa, Artificial Sequence
  4-1BB co-stimulatory domain
KRGRKKLLYIFKQPFMRPVQTTQEEDGCSCRFPEEEEGGCEL

SEQ ID NO: 22 - DNA, 126 bp, Artificial Sequence
  4-1BB co-stimulatory domain
aaacggggcagaaagaaactcctgtatatattcaaacaaccatttatgagaccagtacaaactactcaagaggaagatggctgtagctgccgatttccagaagaagaagaaggaggatgtgaactg

SEQ ID NO: 23 - protein, 242 aa, Artificial Sequence
  alpha CD19 scFv
DIQMTQTTSSLSASLGDRVTISCRASQDISKYLNWYQQKPDGTVKLLIYHTSRLHSGVPSRFSGSGSGTDYSLTISNLEQEDIATYFCQQGNTLPYTFGGGTKLEITGGGGSGGGGSGGGGSEVKLQESGPGLVAPSQSLSVTCTVSGVSLPDYGVSWIRQPPRKGLEWLGVIWGSETTYYNSALKSRLTIIKDNSKSQVFLKMNSLQTDDTAIYYCAKHYYYGGSYAMDYWGQGTSVTVSS

SEQ ID NO: 24 - DNA, 726 bp, Artificial Sequence
  alpha CD19 scFv
gacatccagatgacacagactacatcctccctgtctgcctctctgggagacagagtcaccatcagttgcagggcaagtcaggacattagtaaatatttaaattggtatcagcagaaaccagatggaactgttaaactcctgatctaccatacatcaagattacactcaggagtcccatcaaggttcagtggcagtgggtctggaacagattattctctcaccattagcaacctggagcaagaagatattgccacttacttttgccaacagggtaatacgcttccgtacacgttcggaggggggaccaagctggagatcacaggtggcggtggctcgggcggtggtgggtcgggtggcggcggatctgaggtgaaactgcaggagtcaggacctggcctggtggcgccctcacagagcctgtccgtcacatgcactgtctcaggggtctcattacccgactatggtgtaagctggattcgccagcctccacgaaagggtctggagtggctgggagtaatatggggtagtgaaaccacatactataattcagctctcaaatccagactgaccatcatcaaggacaactccaagagccaagttttcttaaaaatgaacagtctgcaaactgatgacacagccatttactactgtgccaaacattattactacggtggtagctatgctatggactactggggccaaggaacctcagtcaccgtctcctca

SEQ ID NO: 25 - protein, 21 aa, Artificial Sequence
  hCD8L
MALPVTALLLPLALLLHAARP

SEQ ID NO: 26 - DNA, 63 bp, Artificial Sequence
  hCD8L
atggccttaccagtgaccgccttgctcctgccgctggccttgctgctccacgccgccaggccg

SEQ ID NO: 27 - protein, 511 aa, Artificial Sequence
  F58BBz
MALPVTALLLPLALLLHAARPDIQMTQTTSSLSASLGDRVTISCRASQDISKYLNWYQQKPDGTVKLLIYHTSRLHSGVPSRFSGSGSGTDYSLTISNLEQEDIATYFCQQGNTLPYTFGGGTKLEITGGGGSGGGGSGGGGSEVKLQESGPGLVAPSQSLSVTCTVSGVSLPDYGVSWIRQPPRKGLEWLGVIWGSETTYYNSALKSRLTIIKDNSKSQVFLKMNSLQTDDTAIYYCAKHYYYGGSYAMDYWGQGTSVTVSSDDPRPPNPPKPMPNPNPNHPSSSGSFSDADLADGVSGGEGKGGSDGGGSHRKEGEEADAPGVIPGIVGAVVVAVAGAISSFIAYQKKKLCFKENKRGRKKLLYIFKQPFMRPVQTTQEEDGCSCRFPEEEEGGCELRVKFSRSADAPAYKQGQNQLYNELNLGRREEYDVLDKRRGRDPEMGGKPRRKNPQEGLYNELQKDKMAEAYSEIGMKGERRRGKGHDGLYQGLSTATKDTYDALHMQALPPR

SEQ ID NO: 28 - DNA, 1536 bp, Artificial Sequence
  F58BBz
atggccttaccagtgaccgccttgctcctgccgctggccttgctgctccacgccgccaggccggacatccagatgacacagactacatcctccctgtctgcctctctgggagacagagtcaccatcagttgcagggcaagtcaggacattagtaaatatttaaattggtatcagcagaaaccagatggaactgttaaactcctgatctaccatacatcaagattacactcaggagtcccatcaaggttcagtggcagtgggtctggaacagattattctctcaccattagcaacctggagcaagaagatattgccacttacttttgccaacagggtaatacgcttccgtacacgttcggaggggggaccaagctggagatcacaggtggcggtggctcgggcggtggtgggtcgggtggcggcggatctgaggtgaaactgcaggagtcaggacctggcctggtggcgccctcacagagcctgtccgtcacatgcactgtctcaggggtctcattacccgactatggtgtaagctggattcgccagcctccacgaaagggtctggagtggctgggagtaatatggggtagtgaaaccacatactataattcagctctcaaatccagactgaccatcatcaaggacaactccaagagccaagttttcttaaaaatgaacagtctgcaaactgatgacacagccatttactactgtgccaaacattattactacggtggtagctatgctatggactactggggccaaggaacctcagtcaccgtctcctcagacgacccacgaccaccgaacccacccaaaccgatgccaaatccaaaccccaaccaccctagttcctccggtagcttttcagatgctgaccttgcggatggcgtttcaggtggagaaggaaaaggaggcagtgatggtggaggcagccacaggaaagaaggggaagaggccgacgccccaggcgtgatccccgggattgtgggggctgtcgtggtcgccgtggctggagccatctctagcttcattgcttaccagaaaaagaagctatgcttcaaagaaaataaacggggcagaaagaaactcctgtatatattcaaacaaccatttatgagaccagtacaaactactcaagaggaagatggctgtagctgccgatttccagaagaagaagaaggaggatgtgaactgagagtgaagttcagcaggagcgcagacgcccccgcgtacaagcagggccagaaccagctctataacgagctcaatctaggacgaagagaggagtacgatgttttggacaagagacgtggccgggaccctgagatggggggaaagccgagaaggaagaaccctcaggaaggcctgtacaatgaactgcagaaagataagatggcggaggcctacagtgagattgggatgaaaggcgagcgccggaggggcaaggggcacgatggcctttaccagggtctcagtacagccaccaaggacacctacgacgcccttcacatgcaggccctgccccctcgctaa

SEQ ID NO: 29 - protein, 498 aa, Artificial Sequence
  F45BBz
MALPVTALLLPLALLLHAARPDIQMTQTTSSLSASLGDRVTISCRASQDISKYLNWYQQKPDGTVKLLIYHTSRLHSGVPSRFSGSGSGTDYSLTISNLEQEDIATYFCQQGNTLPYTFGGGTKLEITGGGGSGGGGSGGGGSEVKLQESGPGLVAPSQSLSVTCTVSGVSLPDYGVSWIRQPPRKGLEWLGVIWGSETTYYNSALKSRLTIIKDNSKSQVFLKMNSLQTDDTAIYYCAKHYYYGGSYAMDYWGQGTSVTVSSNPNPNHPSSSGSFSDADLADGVSGGEGKGGSDGGGSHRKEGEEADAPGVIPGIVGAVVVAVAGAISSFIAYQKKKLCFKENKRGRKKLLYIFKQPFMRPVQTTQEEDGCSCRFPEEEEGGCELRVKFSRSADAPAYKQGQNQLYNELNLGRREEYDVLDKRRGRDPEMGGKPRRKNPQEGLYNELQKDKMAEAYSEIGMKGERRRGKGHDGLYQGLSTATKDTYDALHMQALPPR

SEQ ID NO: 30 - DNA, 1497 bp, Artificial Sequence
  F45BBz
atggccttaccagtgaccgccttgctcctgccgctggccttgctgctccacgccgccaggccggacatccagatgacacagactacatcctccctgtctgcctctctgggagacagagtcaccatcagttgcagggcaagtcaggacattagtaaatatttaaattggtatcagcagaaaccagatggaactgttaaactcctgatctaccatacatcaagattacactcaggagtcccatcaaggttcagtggcagtgggtctggaacagattattctctcaccattagcaacctggagcaagaagatattgccacttacttttgccaacagggtaatacgcttccgtacacgttcggaggggggaccaagctggagatcacaggtggcggtggctcgggcggtggtgggtcgggtggcggcggatctgaggtgaaactgcaggagtcaggacctggcctggtggcgccctcacagagcctgtccgtcacatgcactgtctcaggggtctcattacccgactatggtgtaagctggattcgccagcctccacgaaagggtctggagtggctgggagtaatatggggtagtgaaaccacatactataattcagctctcaaatccagactgaccatcatcaaggacaactccaagagccaagttttcttaaaaatgaacagtctgcaaactgatgacacagccatttactactgtgccaaacattattactacggtggtagctatgctatggactactggggccaaggaacctcagtcaccgtctcctcaaatccaaaccccaaccaccctagttcctccggtagcttttcagatgctgaccttgcggatggcgtttcaggtggagaaggaaaaggaggcagtgatggtggaggcagccacaggaaagaaggggaagaggccgacgccccaggcgtgatccccgggattgtgggggctgtcgtggtcgccgtggctggagccatctctagcttcattgcttaccagaaaaagaagctatgcttcaaagaaaataaacggggcagaaagaaactcctgtatatattcaaacaaccatttatgagaccagtacaaactactcaagaggaagatggctgtagctgccgatttccagaagaagaagaaggaggatgtgaactgagagtgaagttcagcaggagcgcagacgcccccgcgtacaagcagggccagaaccagctctataacgagctcaatctaggacgaagagaggagtacgatgttttggacaagagacgtggccgggaccctgagatggggggaaagccgagaaggaagaaccctcaggaaggcctgtacaatgaactgcagaaagataagatggcggaggcctacagtgagattgggatgaaaggcgagcgccggaggggcaaggggcacgatggcctttaccagggtctcagtacagccaccaaggacacctacgacgcccttcacatgcaggccctgccccctcgctaa

SEQ ID NO: 31 - protein, 488 aa, Artificial Sequence
  F35BBz
MALPVTALLLPLALLLHAARPDIQMTQTTSSLSASLGDRVTISCRASQDISKYLNWYQQKPDGTVKLLIYHTSRLHSGVPSRFSGSGSGTDYSLTISNLEQEDIATYFCQQGNTLPYTFGGGTKLEITGGGGSGGGGSGGGGSEVKLQESGPGLVAPSQSLSVTCTVSGVSLPDYGVSWIRQPPRKGLEWLGVIWGSETTYYNSALKSRLTIIKDNSKSQVFLKMNSLQTDDTAIYYCAKHYYYGGSYAMDYWGQGTSVTVSSGSFSDADLADGVSGGEGKGGSDGGGSHRKEGEEADAPGVIPGIVGAVVVAVAGAISSFIAYQKKKLCFKENKRGRKKLLYIFKQPFMRPVQTTQEEDGCSCRFPEEEEGGCELRVKFSRSADAPAYKQGQNQLYNELNLGRREEYDVLDKRRGRDPEMGGKPRRKNPQEGLYNELQKDKMAEAYSEIGMKGERRRGKGHDGLYQGLSTATKDTYDALHMQALPPR

SEQ ID NO: 32 - DNA, 1467 bp, Artificial Sequence
  F35BBz
atggccttaccagtgaccgccttgctcctgccgctggccttgctgctccacgccgccaggccggacatccagatgacacagactacatcctccctgtctgcctctctgggagacagagtcaccatcagttgcagggcaagtcaggacattagtaaatatttaaattggtatcagcagaaaccagatggaactgttaaactcctgatctaccatacatcaagattacactcaggagtcccatcaaggttcagtggcagtgggtctggaacagattattctctcaccattagcaacctggagcaagaagatattgccacttacttttgccaacagggtaatacgcttccgtacacgttcggaggggggaccaagctggagatcacaggtggcggtggctcgggcggtggtgggtcgggtggcggcggatctgaggtgaaactgcaggagtcaggacctggcctggtggcgccctcacagagcctgtccgtcacatgcactgtctcaggggtctcattacccgactatggtgtaagctggattcgccagcctccacgaaagggtctggagtggctgggagtaatatggggtagtgaaaccacatactataattcagctctcaaatccagactgaccatcatcaaggacaactccaagagccaagttttcttaaaaatgaacagtctgcaaactgatgacacagccatttactactgtgccaaacattattactacggtggtagctatgctatggactactggggccaaggaacctcagtcaccgtctcctcaggtagcttttcagatgctgaccttgcggatggcgtttcaggtggagaaggaaaaggaggcagtgatggtggaggcagccacaggaaagaaggggaagaggccgacgccccaggcgtgatccccgggattgtgggggctgtcgtggtcgccgtggctggagccatctctagcttcattgcttaccagaaaaagaagctatgcttcaaagaaaataaacggggcagaaagaaactcctgtatatattcaaacaaccatttatgagaccagtacaaactactcaagaggaagatggctgtagctgccgatttccagaagaagaagaaggaggatgtgaactgagagtgaagttcagcaggagcgcagacgcccccgcgtacaagcagggccagaaccagctctataacgagctcaatctaggacgaagagaggagtacgatgttttggacaagagacgtggccgggaccctgagatggggggaaagccgagaaggaagaaccctcaggaaggcctgtacaatgaactgcagaaagataagatggcggaggcctacagtgagattgggatgaaaggcgagcgccggaggggcaaggggcacgatggcctttaccagggtctcagtacagccaccaaggacacctacgacgcccttcacatgcaggccctgccccctcgctaa

SEQ ID NO: 33 - protein, 488 aa, Artificial Sequence
  F35BBz-1
MALPVTALLLPLALLLHAARPDIQMTQTTSSLSASLGDRVTISCRASQDISKYLNWYQQKPDGTVKLLIYHTSRLHSGVPSRFSGSGSGTDYSLTISNLEQEDIATYFCQQGNTLPYTFGGGTKLEITGGGGSGGGGSGGGGSEVKLQESGPGLVAPSQSLSVTCTVSGVSLPDYGVSWIRQPPRKGLEWLGVIWGSETTYYNSALKSRLTIIKDNSKSQVFLKMNSLQTDDTAIYYCAKHYYYGGSYAMDYWGQGTSVTVSSGSFSDADLADGVSGGEGKGGSDGGGSHRKEGEEADAPGVIPGIVGAVVVAVAGAISSFIAYQKKKLCFKENKRGRKKLLYIFKQPFMRPVQTTQEEDGCSCRFPEEEEGGCELRVKFSRSADAPAYQQGQNQLYNELNLGRREEYDVLDKRRGRDPEMGGKPRRKNPQEGLYNELQKDKMAEAYSEIGMKGERRRGKGHDGLYQGLSTATKDTYDALHMQALPPR

SEQ ID NO: 34 - DNA, 1467 bp, Artificial Sequence
  F35BBz-1
atggccttaccagtgaccgccttgctcctgccgctggccttgctgctccacgccgccaggccggacatccagatgacacagactacatcctccctgtctgcctctctgggagacagagtcaccatcagttgcagggcaagtcaggacattagtaaatatttaaattggtatcagcagaaaccagatggaactgttaaactcctgatctaccatacatcaagattacactcaggagtcccatcaaggttcagtggcagtgggtctggaacagattattctctcaccattagcaacctggagcaagaagatattgccacttacttttgccaacagggtaatacgcttccgtacacgttcggaggggggaccaagctggagatcacaggtggcggtggctcgggcggtggtgggtcgggtggcggcggatctgaggtgaaactgcaggagtcaggacctggcctggtggcgccctcacagagcctgtccgtcacatgcactgtctcaggggtctcattacccgactatggtgtaagctggattcgccagcctccacgaaagggtctggagtggctgggagtaatatggggtagtgaaaccacatactataattcagctctcaaatccagactgaccatcatcaaggacaactccaagagccaagttttcttaaaaatgaacagtctgcaaactgatgacacagccatttactactgtgccaaacattattactacggtggtagctatgctatggactactggggccaaggaacctcagtcaccgtctcctcaggtagcttttcagatgctgaccttgcggatggcgtttcaggtggagaaggaaaaggaggcagtgatggtggaggcagccacaggaaagaaggggaagaggccgacgccccaggcgtgatccccgggattgtgggggctgtcgtggtcgccgtggctggagccatctctagcttcattgcttaccagaaaaagaagctatgcttcaaagaaaataaacggggcagaaagaaactcctgtatatattcaaacaaccatttatgagaccagtacaaactactcaagaggaagatggctgtagctgccgatttccagaagaagaagaaggaggatgtgaactgagagtgaagttcagcaggagcgcagacgcccccgcgtaccagcagggccagaaccagctctataacgagctcaatctaggacgaagagaggagtacgatgttttggacaagagacgtggccgggaccctgagatggggggaaagccgagaaggaagaaccctcaggaaggcctgtacaatgaactgcagaaagataagatggcggaggcctacagtgagattgggatgaaaggcgagcgccggaggggcaaggggcacgatggcctttaccagggtctcagtacagccaccaaggacacctacgacgcccttcacatgcaggccctgccccctcgctaa

SEQ ID NO: 35 - protein, 186 aa, Artificial Sequence
  CD99 WT
MARAAMEAAATVVLALALLGAAARGAAEQKLISEEDLNSDDFNLGDALEDPNMKPTPKAPTPKKPSGGFDLEDALPGGGGGGAGEKPGNRPQPDPKPPRPHGDSGGISDSDLADAAGQGGGGAGRRGSGDEGGHGGAGGAEPEGTPQGLVPGVVAAVVAAVAGAVSSFVAYQRRRLCFREGGSAPV

SEQ ID NO: 36 - protein, 187 aa, Artificial Sequence
  CD99 TM mutant
MARAAMEAAATVVLALALLGAAARGAAEQKLISEEDLNSDDFNLGDALEDPNMKPTPKAPTPKKPSGGFDLEDALPGGGGGGAGEKPGNRPQPDPKPPRPHGDSGGISDSDLADAAGQGGGGAGRRGSGDEGGHGGAGGAEPEGTPQGALIVLGGVAGLLLFIGLGIFFCAYQRRRLCFREGGSAPV

SEQ ID NO: 37 - protein, 177 aa, Artificial Sequence
  CD99 Cyt mutant
MARAAMEAAATVVLALALLGAAARGAAEQKLISEEDLNSDDFNLGDALEDPNMKPTPKAPTPKKPSGGFDLEDALPGGGGGGAGEKPGNRPQPDPKPPRPHGDSGGISDSDLADAAGQGGGGAGRRGSGDEGGHGGAGGAEPEGTPQGLVPGVVAAVVAAVAGAVSSFVVRCRHRRR

SEQ ID NO: 38 - protein, 189 aa, Artificial Sequence
  CD99 TMrst-S mutant
MARAAMEAAATVVLALALLGAAARGAAEQKLISEEDLNSDDFNLGDALEDPNMKPTPKAPTPKKPSGGFDLEDALPGGGGGGAGEKPGNRPQPDPKPPRPHGDSGGISDSDLADAAGQGGGGAGRRGSGDEGGHGGAGGAEPEGTPQGALIVLGGVAGLLLFIGLGAVSSFVAYQRRRLCFREGGSAPV

SEQ ID NO: 39 - protein, 188 aa, Artificial Sequence
  CD99 TMrst-L mutant
MARAAMEAAATVVLALALLGAAARGAAEQKLISEEDLNSDDFNLGDALEDPNMKPTPKAPTPKKPSGGFDLEDALPGGGGGGAGEKPGNRPQPDPKPPRPHGDSGGISDSDLADAAGQGGGGAGRRGSGDEGGHGGAGGAEPEGTPQGALIVLGGVAGLVAAVAGAVSSFVAYQRRRLCFREGGSAPV

SEQ ID NO: 40 - protein, 180 aa, Artificial Sequence
  CD99 CytJuxt mutant
MARAAMEAAATVVLALALLGAAARGAAEQKLISEEDLNSDDFNLGDALEDPNMKPTPKAPTPKKPSGGFDLEDALPGGGGGGAGEKPGNRPQPDPKPPRPHGDSGGISDSDLADAAGQGGGGAGRRGSGDEGGHGGAGGAEPEGTPQGLVPGVVAAVVAAVAGAVSSFVAYQRRRLCFRE

SEQ ID NO: 41 - protein, 486 aa, Artificial Sequence
  hCD19BBz
MALPVTALLLPLALLLHAARPDIQMTQTTSSLSASLGDRVTISCRASQDISKYLNWYQQKPDGTVKLLIYHTSRLHSGVPSRFSGSGSGTDYSLTISNLEQEDIATYFCQQGNTLPYTFGGGTKLEITGGGGSGGGGSGGGGSEVKLQESGPGLVAPSQSLSVTCTVSGVSLPDYGVSWIRQPPRKGLEWLGVIWGSETTYYNSALKSRLTIIKDNSKSQVFLKMNSLQTDDTAIYYCAKHYYYGGSYAMDYWGQGTSVTVSSTTTPAPRPPTPAPTIASQPLSLRPEACRPAAGGAVHTRGLDFACDIYIWAPLAGTCGVLLLSLVITLYCKRGRKKLLYIFKQPFMRPVQTTQEEDGCSCRFPEEEEGGCELRVKFSRSADAPAYKQGQNQLYNELNLGRREEYDVLDKRRGRDPEMGGKPRRKNPQEGLYNELQKDKMAEAYSEIGMKGERRRGKGHDGLYQGLSTATKDTYDALHMQALPPR

SEQ ID NO: 42 - DNA, 1461 bp, Artificial Sequence
  hCD19BBz
atggccttaccagtgaccgccttgctcctgccgctggccttgctgctccacgccgccaggccggacatccagatgacacagactacatcctccctgtctgcctctctgggagacagagtcaccatcagttgcagggcaagtcaggacattagtaaatatttaaattggtatcagcagaaaccagatggaactgttaaactcctgatctaccatacatcaagattacactcaggagtcccatcaaggttcagtggcagtgggtctggaacagattattctctcaccattagcaacctggagcaagaagatattgccacttacttttgccaacagggtaatacgcttccgtacacgttcggaggggggaccaagctggagatcacaggtggcggtggctcgggcggtggtgggtcgggtggcggcggatctgaggtgaaactgcaggagtcaggacctggcctggtggcgccctcacagagcctgtccgtcacatgcactgtctcaggggtctcattacccgactatggtgtaagctggattcgccagcctccacgaaagggtctggagtggctgggagtaatatggggtagtgaaaccacatactataattcagctctcaaatccagactgaccatcatcaaggacaactccaagagccaagttttcttaaaaatgaacagtctgcaaactgatgacacagccatttactactgtgccaaacattattactacggtggtagctatgctatggactactggggccaaggaacctcagtcaccgtctcctcaaccacgacgccagcgccgcgaccaccaacaccggcgcccaccatcgcgtcgcagcccctgtccctgcgcccagaggcgtgccggccagcggcggggggcgcagtgcacacgagggggctggacttcgcctgtgatatctacatctgggcgcccttggccgggacttgtggggtccttctcctgtcactggttatcaccctttactgcaaacggggcagaaagaaactcctgtatatattcaaacaaccatttatgagaccagtacaaactactcaagaggaagatggctgtagctgccgatttccagaagaagaagaaggaggatgtgaactgagagtgaagttcagcaggagcgcagacgcccccgcgtacaagcagggccagaaccagctctataacgagctcaatctaggacgaagagaggagtacgatgttttggacaagagacgtggccgggaccctgagatggggggaaagccgagaaggaagaaccctcaggaaggcctgtacaatgaactgcagaaagataagatggcggaggcctacagtgagattgggatgaaaggcgagcgccggaggggcaaggggcacgatggcctttaccagggtctcagtacagccaccaaggacacctacgacgcccttcacatgcaggccctgccccctcgctaa

SEQ ID NO: 43 - protein, 496 aa, Artificial Sequence
  F8TJBBz
MALPVTALLLPLALLLHAARPDIQMTQTTSSLSASLGDRVTISCRASQDISKYLNWYQQKPDGTVKLLIYHTSRLHSGVPSRFSGSGSGTDYSLTISNLEQEDIATYFCQQGNTLPYTFGGGTKLEITGGGGSGGGGSGGGGSEVKLQESGPGLVAPSQSLSVTCTVSGVSLPDYGVSWIRQPPRKGLEWLGVIWGSETTYYNSALKSRLTIIKDNSKSQVFLKMNSLQTDDTAIYYCAKHYYYGGSYAMDYWGQGTSVTVSSTTTPAPRPPTPAPTIASQPLSLRPEACRPAAGGAVHTRGLDADAPGVIPGIVGAVVVAVAGAISSFIAYQKKKLCFKENKRGRKKLLYIFKQPFMRPVQTTQEEDGCSCRFPEEEEGGCELRVKFSRSADAPAYKQGQNQLYNELNLGRREEYDVLDKRRGRDPEMGGKPRRKNPQEGLYNELQKDKMAEAYSEIGMKGERRRGKGHDGLYQGLSTATKDTYDALHMQALPPR

SEQ ID NO: 44 - DNA, 1491 bp, Artificial Sequence
  F8TJBBz
atggccttaccagtgaccgccttgctcctgccgctggccttgctgctccacgccgccaggccggacatccagatgacacagactacatcctccctgtctgcctctctgggagacagagtcaccatcagttgcagggcaagtcaggacattagtaaatatttaaattggtatcagcagaaaccagatggaactgttaaactcctgatctaccatacatcaagattacactcaggagtcccatcaaggttcagtggcagtgggtctggaacagattattctctcaccattagcaacctggagcaagaagatattgccacttacttttgccaacagggtaatacgcttccgtacacgttcggaggggggaccaagctggagatcacaggtggcggtggctcgggcggtggtgggtcgggtggcggcggatctgaggtgaaactgcaggagtcaggacctggcctggtggcgccctcacagagcctgtccgtcacatgcactgtctcaggggtctcattacccgactatggtgtaagctggattcgccagcctccacgaaagggtctggagtggctgggagtaatatggggtagtgaaaccacatactataattcagctctcaaatccagactgaccatcatcaaggacaactccaagagccaagttttcttaaaaatgaacagtctgcaaactgatgacacagccatttactactgtgccaaacattattactacggtggtagctatgctatggactactggggccaaggaacctcagtcaccgtctcctcaaccacgacgccagcgccgcgaccaccaacaccggcgcccaccatcgcgtcgcagcccctgtccctgcgcccagaggcgtgccggccagcggcggggggcgcagtgcacacgagggggctggacgccgacgccccaggcgtgatccccgggattgtgggggctgtcgtggtcgccgtggctggagccatctctagcttcattgcttaccagaaaaagaagctatgcttcaaagaaaataaacggggcagaaagaaactcctgtatatattcaaacaaccatttatgagaccagtacaaactactcaagaggaagatggctgtagctgccgatttccagaagaagaagaaggaggatgtgaactgagagtgaagttcagcaggagcgcagacgcccccgcgtacaagcagggccagaaccagctctataacgagctcaatctaggacgaagagaggagtacgatgttttggacaagagacgtggccgggaccctgagatggggggaaagccgagaaggaagaaccctcaggaaggcctgtacaatgaactgcagaaagataagatggcggaggcctacagtgagattgggatgaaaggcgagcgccggaggggcaaggggcacgatggcctttaccagggtctcagtacagccaccaaggacacctacgacgcccttcacatgcaggccctgccccctcgctaa